European Patent Specification EP 3 315 599 B1, published August 26, 2026. Title: Oral tumor vaccine. Applicant: NATIONAL UNIVERSITY CORPORATION KOBE UNIVERSITY OSAKA UNIVERSITY. Application JP2015-128034. The sequence listing filed with the application follows.

SEQUENCE LISTING (26 sequences)

SEQ ID NO: 1 - protein, 323 aa, Mus musculus
PSQASSGQARMFPNAPYLPSCLESQPTIRNQGYSTVTFDGAPSYGHTPSHHAAQFPNHSFKHEDPMGQQGSLGEQQYSVPPPVYGCHTPTDSCTGSQALLLRTPYSSDNLYQMTSQLECMTWNQMNLGATLKGMAAGSSSSVKWTEGQSNHGIGYESENHTAPILCGAQYRIHTHGVFRGIQDVRRVSGVAPTLVRSASETSEKRPFMCAYPGCNKRYFKLSHLQMHSRKHTGEKPYQCDFKDCERRFSRSDQLKRHQRRHTGVKPFQCKTCQRKFSRSDHLKTHTRTHTGKTSEKPFSCRWHSCQKKFARSDELVRHHNMHQ

SEQ ID NO: 2 - DNA, 985 bp, Mus musculus
ctcgagccgtcccaggcgtcgtcgggccaggcgaggatgttcccgaacgcgccctacctgcccagctgcctggagtcccagccgacgatccgcaaccagggctactccaccgtgacgttcgacggcgccccgtcctacggccacacgcccagccaccacgccgcccagttcccgaaccacagcttcaagcacgaagaccccatgggccagcagggcagcctcggcgaacagcagtacagcgtgccgccgccggtctacggctgccacaccccgaccgactcctgcacgggctcccaggccctgctcctgcgtacgccgtactcctccgacaacctctaccagatgacctcccagctggagtgcatgacctggaaccagatgaacctgggcgccacgctgaagggaatggccgcggggtcgtcgagctccgtcaagtggaccgaaggccagtccaaccacggcatcggctacgagtccgagaaccacaccgcgccgatcctgtgcggagcccagtaccgcatccacacgcacggcgtcttccgcggcatccaggacgtccggcgcgtctccggcgtcgcgccgaccctggtgcggtccgcctccgagacctccgagaagcgcccgttcatgtgcgcctacccgggctgcaacaagcgctacttcaagctctcgcacctgcagatgcactcccggaagcacaccggcgagaagccgtaccagtgcgacttcaaggactgcgaacgccgcttctcgcgcagcgaccagctgaagcgccaccagcgtaggcacaccggcgtgaagcccttccagtgcaagacctgccagcgcaagttctcccgcagcgaccacctcaagacgcacacccgcacccacaccggcaagacgtccgagaagccgttctcgtgccgctggcacagctgccagaagaagttcgcccgcagcgacgagctcgtgcgccaccacaacatgcaccagtgaagcatgc

SEQ ID NO: 3 - DNA, 22 bp, Artificial
  Primer for GL-BP (glt-f)
ggggtgctgatatattggtttg

SEQ ID NO: 4 - DNA, 31 bp, Artificial
  Primer for GL-BP (glt-r)
gctcgagctcggaaacagacaggccgaagtt

SEQ ID NO: 5 - DNA, 6 bp, Artificial
  Recognition sequence for XhoI
ctcgag

SEQ ID NO: 6 - DNA, 6 bp, Artificial
  Recognition sequence for SphI
gcatgc

SEQ ID NO: 7 - DNA, 24 bp, Artificial
  Primer for WT1 (WT1-f)
cgctcgagccgtcccaggcgtcgt

SEQ ID NO: 8 - DNA, 30 bp, Artificial
  Primer for WT1 (WT1-r2)
gcgcatgctcactcgccggtgtgcttccgg

SEQ ID NO: 9 - DNA, 36 bp, Artificial
  Primer  (Infusion-F)
ggaaaactgtccatagatggcgaggcgaacgccacg

SEQ ID NO: 10 - DNA, 36 bp, Artificial
  Primer  (Infusion-R)
tttcatctgtgcatagtgctgcaaggcgattaagtt

SEQ ID NO: 11 - DNA, 23 bp, Artificial
  Primer  (410, 420-F)
acgatccgcaaccagggctactc

SEQ ID NO: 12 - DNA, 23 bp, Artificial
  Primer  (410-R)
ggtgcgagagcttgaagtagcgc

SEQ ID NO: 13 - DNA, 22 bp, Artificial
  Primer  (420-R)
gtcgctgcgggcgaacttcttc

SEQ ID NO: 14 - protein, 323 aa, Homo sapiens
PSQASSGQARMFPNAPYLPSCLESQPAIRNQGYSTVTFDGTPSYGHTPSHHAAQFPNHSFKHEDPMGQQGSLGEQQYSVPPPVYGCHTPTDSCTGSQALLLRTPYSSDNLYQMTSQLECMTWNQMNLGATLKGVAAGSSSSVKWTEGQSNHSTGYESDNHTTPILCGAQYRIHTHGVFRGIQDVRRVPGVAPTLVRSASETSEKRPFMCAYPGCNKRYFKLSHLQMHSRKHTGEKPYQCDFKDCERRFSRSDQLKRHQRRHTGVKPFQCKTCQRKFSRSDHLKTHTRTHTGKTSEKPFSCRWPSCQKKFARSDELVRHHNMHQ

SEQ ID NO: 15 - DNA, 973 bp, Homo sapiens
ccgtcccaggcgtcgtcgggccaggcgaggatgttcccgaacgcgccctacctgcccagctgcctggagtcccagccggcgatccgcaaccagggctactccaccgtgacgttcgacggcaccccgtcctacggccacacgcccagccaccacgccgcccagttcccgaaccacagcttcaagcacgaagaccccatgggccagcagggcagcctcggcgaacagcagtacagcgtgccgccgccggtctacggctgccacaccccgaccgactcctgcacgggctcccaggccctgctcctgcgtacgccgtactcctccgacaacctctaccagatgacctcccagctggagtgcatgacctggaaccagatgaacctgggcgccacgctgaagggagtcgccgcggggtcgtcgagctccgtcaagtggaccgaaggccagtccaaccactccaccggctacgagtccgacaaccacaccacgccgatcctgtgcggagcccagtaccgcatccacacgcacggcgtcttccgcggcatccaggacgtccggcgcgtccccggcgtcgcgccgaccctggtgcggtccgcctccgagacctccgagaagcgcccgttcatgtgcgcctacccgggctgcaacaagcgctacttcaagctctcgcacctgcagatgcactcccggaagcacaccggcgagaagccgtaccagtgcgacttcaaggactgcgaacgccgcttctcgcgcagcgaccagctgaagcgccaccagcgtaggcacaccggcgtgaagcccttccagtgcaagacctgccagcgcaagttctcccgcagcgaccacctcaagacgcacacccgcacccacaccggcaagacgtccgagaagccgttctcgtgccgctggcccagctgccagaagaagttcgcccgcagcgacgagctcgtgcgccaccacaacatgcaccagtgaa

SEQ ID NO: 16 - protein, 323 aa, Homo sapiens
PSQASSGQARMFPNAPYLPSCLESQPAIRNQGYSTVTFDGTPSYGHTPSHHAAQFPNHSFKHEDPMGQQGSLGEQQYSVPPPVYGCHTPTDSCTGSQALLLRTPYSSDNLYQMTSQLECYTWNQMNLGATLKGVAAGSSSSVKWTEGQSNHSTGYESDNHTTPILCGAQYRIHTHGVFRGIQDVRRVPGVAPTLVRSASETSEKRPFMCAYPGCNKRYFKLSHLQMHSRKHTGEKPYQCDFKDCERRFSRSDQLKRHQRRHTGVKPFQCKTCQRKFSRSDHLKTHTRTHTGKTSEKPFSCRWPSCQKKFARSDELVRHHNMHQ

SEQ ID NO: 17 - DNA, 973 bp, Homo sapiens
ccgtcccaggcgtcgtcgggccaggcgaggatgttcccgaacgcgccctacctgcccagctgcctggagtcccagccggcgatccgcaaccagggctactccaccgtgacgttcgacggcaccccgtcctacggccacacgcccagccaccacgccgcccagttcccgaaccacagcttcaagcacgaagaccccatgggccagcagggcagcctcggcgaacagcagtacagcgtgccgccgccggtctacggctgccacaccccgaccgactcctgcacgggctcccaggccctgctcctgcgtacgccgtactcctccgacaacctctaccagatgacctcccagctggagtgctacacctggaaccagatgaacctgggcgccacgctgaagggagtcgccgcggggtcgtcgagctccgtcaagtggaccgaaggccagtccaaccactccaccggctacgagtccgacaaccacaccacgccgatcctgtgcggagcccagtaccgcatccacacgcacggcgtcttccgcggcatccaggacgtccggcgcgtccccggcgtcgcgccgaccctggtgcggtccgcctccgagacctccgagaagcgcccgttcatgtgcgcctacccgggctgcaacaagcgctacttcaagctctcgcacctgcagatgcactcccggaagcacaccggcgagaagccgtaccagtgcgacttcaaggactgcgaacgccgcttctcgcgcagcgaccagctgaagcgccaccagcgtaggcacaccggcgtgaagcccttccagtgcaagacctgccagcgcaagttctcccgcagcgaccacctcaagacgcacacccgcacccacaccggcaagacgtccgagaagccgttctcgtgccgctggcccagctgccagaagaagttcgcccgcagcgacgagctcgtgcgccaccacaacatgcaccagtgaa

SEQ ID NO: 18 - protein, 16 aa, Artificial Sequence
  T cell epitope np332
KRYFKLSHLQMHSRKH

SEQ ID NO: 19 - protein, 9 aa, Artificial Sequence
  T cell epitope np126
RMFPNAPYL

SEQ ID NO: 20 - protein, 9 aa, Artificial Sequence
  T cell epitope n187
SLGEQQYSV

SEQ ID NO: 21 - protein, 9 aa, Artificial Sequence
  T cell epitope n235
CMTWNQMNL

SEQ ID NO: 22 - protein, 449 aa, Mus musculus
MGSDVRDLNALLPAVSSLGGGGGGCGLPVSGARQWAPVLDFAPPGASAYGSLGGPAPPPAPPPPPPPPHSFIKQEPSWGGAEPHEEQCLSAFTLHFSGQFTGTAGACRYGPFGPPPPSQASSGQARMFPNAPYLPSCLESQPTIRNQGYSTVTFDGAPSYGHTPSHHAAQFPNHSFKHEDPMGQQGSLGEQQYSVPPPVYGCHTPTDSCTGSQALLLRTPYSSDNLYQMTSQLECMTWNQMNLGATLKGMAAGSSSSVKWTEGQSNHGIGYESENHTAPILCGAQYRIHTHGVFRGIQDVRRVSGVAPTLVRSASETSEKRPFMCAYPGCNKRYFKLSHLQMHSRKHTGEKPYQCDFKDCERRFSRSDQLKRHQRRHTGVKPFQCKTCQRKFSRSDHLKTHTRTHTGKTSEKPFSCRWHSCQKKFARSDELVRHHNMHQRNMTKLHVAL

SEQ ID NO: 23 - protein, 449 aa, Homo sapiens
MGSDVRDLNALLPAVPSLGGGGGCALPVSGAAQWAPVLDFAPPGASAYGSLGGPAPPPAPPPPPPPPPHSFIKQEPSWGGAEPHEEQCLSAFTVHFSGQFTGTAGACRYGPFGPPPPSQASSGQARMFPNAPYLPSCLESQPAIRNQGYSTVTFDGTPSYGHTPSHHAAQFPNHSFKHEDPMGQQGSLGEQQYSVPPPVYGCHTPTDSCTGSQALLLRTPYSSDNLYQMTSQLECMTWNQMNLGATLKGVAAGSSSSVKWTEGQSNHSTGYESDNHTTPILCGAQYRIHTHGVFRGIQDVRRVPGVAPTLVRSASETSEKRPFMCAYPGCNKRYFKLSHLQMHSRKHTGEKPYQCDFKDCERRFSRSDQLKRHQRRHTGVKPFQCKTCQRKFSRSDHLKTHTRTHTGKTSEKPFSCRWPSCQKKFARSDELVRHHNMHQRNMTKLQLAL

SEQ ID NO: 24 - DNA, 30 bp, Artificial Sequence
  Primer F:430
atgacctcccagctggagtgcatgacctgg

SEQ ID NO: 25 - DNA, 30 bp, Artificial Sequence
  Primer F:440
atgacctcccagctggagtgctacacctgg

SEQ ID NO: 26 - DNA, 32 bp, Artificial Sequence
  Primer R: 430, 440
ccagctgccagaagaagttcgcccgcagcgac